European Patent Application EP 4 183 797 A1, published May 24, 2023. Title: CD47 binder and liposome complex for treatment cancer. Applicant: ForBioKorea Co., Ltd. The sequence listing filed with the application follows.

SEQUENCE LISTING (38 sequences)

SEQ ID NO: 1 - protein, 119 aa, Artificial Sequence
  CD47 binder SV1
MEEELQIIQPDKSVSVAAGESAILHCTITSLFPVGPIQWFRGAGPARVLIYNQRQGPFPRVTTVSETTKRENMDFSISISNITPADAGTYYCIKFRKGSPDTEFKSGAGTELSVRAKPS

SEQ ID NO: 2 - protein, 119 aa, Artificial Sequence
  CD47 binder SV4
MEEELQIIQPDLSVSVAAGESAILHCTITSLFPVGPIQWFRGAGPARVLIYNQRQGPFPRVTTVSETTKRENMDFSISISNITPADAGTYYCIKFRKGSPDTEFLSGAGTELSVRAKPS

SEQ ID NO: 3 - protein, 242 aa, Artificial Sequence
  T001
MVFSIKEPFSIVTDCDEVLTDISPLWVHKIQQNADYFGKYFDLSKLEGLEFGTFEHYQTVLSRPEFHLNKWLRKENLVLSDEEEKELFERFYSLYDNDEFYEDCMPTKMCEGIYKLSLQKFVDKIYVVTRTSEGTKEGKRKFIETFLNSNKVEIIFVGKNEKKSDYIKNLKNVKMIVEDELSNINDIVENCNDGFEEVDTYIPSTGYNNKDIDGFNENLMKKGFNAVPYVIIERPETEEKAV

SEQ ID NO: 4 - DNA, 177 bp, Artificial Sequence
  5'-UTR sequence
ttggtcgtgaggcactgggcaggtaagtatcaaggttacaagacaggtttaaggagaccaatagaaactgggcttgtcgagacagagaagactcttgcgtttctgataggcacctattggtcttactgacatccactttgcctttctctccacaggtgtccactcccagttcaatta

SEQ ID NO: 5 - DNA, 259 bp, Artificial Sequence
  3'-UTR sequence
gaattcacgcgtcgagcatgcatctagggcggccaattccgcccctctcccccccccccctctccctcccccccccctaacgttactggccgaagccgcttggaataaggccggtgtgcgtttgtctatatgttattttccaccatattgccgtcttttggcaatgtgagggcccggaaacctggccctgtcttcttgacgagcattcctaggggtctttcccctctcgccaaaggaatgcaaggtctgttgaatgtcg

SEQ ID NO: 6 - DNA, 177 bp, Artificial Sequence; identical to SEQ ID NO: 4
  5'-UTR sequence

SEQ ID NO: 7 - DNA, 177 bp, Artificial Sequence; identical to SEQ ID NO: 4
  5'-UTR sequence

SEQ ID NO: 8 - DNA, 328 bp, Artificial Sequence
  3'-UTR sequence
gactagtgcatcacatttaaaagcatctcagcctaccatgagaataagagaaagaaaatgaagatcaatagcttattcatctctttttctttttcgttggtgtaaagccaacaccctgtctaaaaaacataaatttctttaatcattttgcctcttttctctgtgcttcaattaataaaaaatggaaagaacctagatctaaaaaaaaaaaaaaaaaaaaaaaaaaaaaaaaaaaaaaaaaaaaaaaaaaaaaaaaaaaaaaaatgcatcccccccccccccccccccccccccccccccaaaggctcttttcagagccaccagaatt

SEQ ID NO: 9 - DNA, 177 bp, Artificial Sequence; identical to SEQ ID NO: 4
  5'-UTR sequence

SEQ ID NO: 10 - DNA, 328 bp, Artificial Sequence; identical to SEQ ID NO: 8
  3'-UTR sequence

SEQ ID NO: 11 - DNA, 74 bp, Artificial Sequence
  5'-UTR sequence
gggtcccgcagtcggcgtccagcggctctgcttgttcgtgtgtgtgtcgttgcaggccttattcaagcttgagg

SEQ ID NO: 12 - DNA, 328 bp, Artificial Sequence; identical to SEQ ID NO: 8
  3'-UTR sequence

SEQ ID NO: 13 - DNA, 83 bp, Artificial Sequence
  5'-UTR sequence
cttcctactcaggctttatacaaagaccaagaggtacaggtgcaagggagagaagaagagtaagaagaaatataagagccacc

SEQ ID NO: 14 - DNA, 101 bp, Artificial Sequence
  3'-UTR sequence
ttaattaagctgccttctgcggggcttgccttctggccatgcccttcttctctcccttgcacctgtacctcttggtctttgaataaagcctgagtaggaag

SEQ ID NO: 15 - DNA, 25 bp, Artificial Sequence
  5'-UTR sequence
agtaagaagaaatataagagccacc

SEQ ID NO: 16 - DNA, 101 bp, Artificial Sequence; identical to SEQ ID NO: 14
  3'-UTR sequence

SEQ ID NO: 17 - DNA, 14 bp, Artificial Sequence
  5'-UTR sequence
gggagactgccacc

SEQ ID NO: 18 - DNA, 101 bp, Artificial Sequence; identical to SEQ ID NO: 14
  3'-UTR sequence

SEQ ID NO: 19 - DNA, 14 bp, Artificial Sequence
  5'-UTR sequence
gggagactgccaag

SEQ ID NO: 20 - DNA, 101 bp, Artificial Sequence; identical to SEQ ID NO: 14
  3'-UTR sequence

SEQ ID NO: 21 - DNA, 6 bp, Artificial Sequence
  5'-UTR sequence
gctagc

SEQ ID NO: 22 - DNA, 101 bp, Artificial Sequence; identical to SEQ ID NO: 14
  3'-UTR sequence

SEQ ID NO: 23 - protein, 18 aa, Artificial Sequence
  Nucleoplasmin NLS sequence
KRPAATKKAGQAKKKKLD

SEQ ID NO: 24 - protein, 25 aa, Artificial Sequence
  Poxvirus MLS sequence
KISVYLTAAVVGFVAYGILKWYRGT

SEQ ID NO: 25 - protein, 503 aa, Unknown
  Human Sirpa
MEPAGPAPGRLGPLLCLLLAASCAWSGVAGEEELQVIQPDKSVSVAAGESAILHCTVTSLIPVGPIQWFRGAGPARELIYNQKEGHFPRVTTVSESTKRENMDFSISISNITPADAGTYYCVKFRKGSPDTEFKSGAGTELSVRAKPSAPVVSGPAARATPQHTVSFTCESHGFSPRDITLKWFKNGNELSDFQTNVDPVGESVSYSIHSTAKVVLTREDVHSQVICEVAHVTLQGDPLRGTANLSETIRVPPTLEVTQQPVRAENQVNVTCQVRKFYPQRLQLTWLENGNVSRTETASTVTENKDGTYNWMSWLLVNVSAHRDDVKLTCQVEHDGQPAVSKSHDLKVSAHPKEQGSNTAAENTGSNERNIYIVVGVVCTLLVALLMAALYLVRIRQKKAQGSTSSTRLHEPEKNAREITQDTNDITYADLNLPKGKKPAPQAAEPNNHTEYASIQTSPQPASEDTLTYADLDMVHLNRTPKQPAPKPEPSFSEYASVQVPRK

SEQ ID NO: 26 - DNA, 357 bp, Unknown
  Human Sirpa DNA sequence
ggtgaggaggagctgcaggtgattcagcctgacaagtccgtatcagttgcagctggagagtcggccattctgcactgcactgtgacctccctgatccctgtggggcccatccagtggttcagaggagctggaccagcccgggaattaatctacaatcaaaaagaaggccacttcccccgggtaacaactgtttcagagtccacaaagagagaaaacatggacttttccatcagcatcagtaacatcaccccagcagatgccggcacctactactgtgtgaagttccggaaagggagccctgacacggagtttaagtctggagcaggcactgagctgtctgtgcgtgccaaaccctct

SEQ ID NO: 27 - DNA, 354 bp, Artificial Sequence
  SV1 DNA sequence
gaagaggaactgcagattattcagccggacaagtccgtaagcgttgcagctggcgagagcgccattctgcactgcactattacctccctgtttccggtgggcccgatccagtggttccgtggcgctggcccagcccgtgtgctgatctacaatcaacgtcagggcccgttcccgcgtgtaaccactgttagcgagaccaccaagcgtgaaaacatggacttttccatcagcatcagcaacatcaccccagcagatgccggcacctactactgtattaagttccgtaaaggcagccctgacacggagtttaagtctggcgcaggcactgagctgtctgtgcgtgccaaaccgtct

SEQ ID NO: 28 - DNA, 33 bp, Artificial Sequence
  KKtoLL11_F1 Primer
gattattcagccggacctgtccgtaagcgttgc

SEQ ID NO: 29 - DNA, 33 bp, Artificial Sequence
  KKtoLL11_R1 Primer
gcaacgcttacggacaggtccggctgaataatc

SEQ ID NO: 30 - DNA, 27 bp, Artificial Sequence
  KKtoLL104_F2 Primer
ctgacacggagtttctgtctggcgcag

SEQ ID NO: 31 - DNA, 27 bp, Artificial Sequence
  KKtoLL104_R2 Primer
ctgcgccagacagaaactccgtgtcag

SEQ ID NO: 32 - protein, 198 aa, Unknown
  NT5M
MGGRALRVLVDMDGVLADFEGGFLRKFRARFPDQPFIALEDRRGFWVSEQYGRLRPGLSEKAISIWESKNFFFELEPLPGAVEAVKEMASLQNTDVFICTSPIKMFKYCPYEKYAWVEKYFGPDFLEQIVLTRDKTVVSADLLIDDRPDITGAEPTPSWEHVLFTACHNQHLQLQPPRRRLHSWADDWKAILDSKRPC

SEQ ID NO: 33 - RNA, 25 nt, Artificial Sequence
  siT001-1 sense
cgagaagaagucagauuacaucaag

SEQ ID NO: 34 - RNA, 25 nt, Artificial Sequence
  siT001-1 antisense
cuugauguaaucugacuucuucucg

SEQ ID NO: 35 - RNA, 25 nt, Artificial Sequence
  siT001-2 sense
cgcaaauucauugaaaccuuccuga

SEQ ID NO: 36 - RNA, 25 nt, Artificial Sequence
  siT001-2 antisense
ucaggaagguuucaaugaauuugcg

SEQ ID NO: 37 - DNA, 32 bp, Artificial Sequence
  Forward Primer for PCR
gtgcttctgacacaacagtctcgaacttaagc

SEQ ID NO: 38 - DNA, 32 bp, Artificial Sequence
  Reverse Primer for PCR
gaagcggccgccttcctactcaggctttattc